European Patent Application EP 4 644 377 A1, published November 5, 2025. Title: LIPID COMPOUND FOR GENE DELIVERY AND LIPID NANOPARTICLE COMPRISING SAME. Applicant: Nanjing CybernaX Biomedical Technology Co., Ltd. Application CN. The sequence listing filed with the application follows.

SEQUENCE LISTING (2 sequences)

SEQ ID NO: 1 - RNA, 2074 nt, synthetic construct
  source 1..2074: mol_type = other RNA
aataaactagtattcttctggtccccacagactcagagagaacccgccaccatggagctgctgatcctgaaggccaacgctatcaccaccatcctgaccgccgtgaccttctgcttcgcctctggccagaacataacagaggaattctaccagtctacctgttctgctgtttccaagggctacctgagcgccctgcggacaggctggtacaccagcgtgatcacaatcgagctgtctaatatcaaggagaacaagtgcaatggtacagatgccaaggtgaagctgatcaagcaggagctagacaagtacaagaatgccgtgaccgaactgcagctcctgatgcagagcacacccccctgtaacaacagagccagaagggaactgccacggtttatgaactacaccctgaacaatgccaagaagacaaacgtgaccctctctaagaaaagaaagcgcagattcctcggcttcctgctgggcgtgggaagcgcctgcgccagcggagtggccgtgtctaaagtgctgcacctggaaggcgaggtgaacaagattaagagcgctctgctgagcaccaacaaggccgtcgtgtccctgagcaatggagtgtccgtgctgaccatcaaggtgctggatctgaaaaactacattgacaagcaactgctgcctatcgtgaacaaacaaagctgtagcatcagcaatatcgaaacagtgatcgagttccagcaaaagaacaaccggctgctggagatcacaagagaattcagcgtcaatgctggcgtgaccacccctgtgagcacctacatgctgaccaacagcgagctgctgagcctgataaatgacatgcctatcacaaacgatcagaaaaagcttatgagcaacaacgtgcagatcgtgcggcagcagagctacagcatcatgtctatcatcaaggaagaagtgctggcctacgtggtccagctgcctctgtatggcgtgatcgacaccccttgctggaagctgcacaccagccctctgtgtacaaccaacacaaaggaaggctctaacatctgcctgaccagaacggatagaggctggtattgcgacaacgccggcagcgtgtcctttttcccccaggccgagacatgcaaggtgcagtctaacagagtgttctgtgataccatgaacagcctgaccctgccttctgagatcaacctgtgcaacgtcgacatcttcaaccccaagtacgattgcaagatcatgaccagcaaaacagacgtgtccagcagcgtgattacatctctgggagccatcgtgagctgctacggaaagaccaagtgcacagctagcaacaaaaatagaggcatcatcaaaacctttagcaacggctgcgactacgtgagcaacaaaggcatggacaccgtgagcgttggcaacaccctatactacgtgaacaaacaggagggcaagtccctgtacgtcaagggcgagcctatcatcaacttctacgaccccctggtgtttcctagcagcgagttcgacgccagcatcagccaggtgaacgagaagatcaaccagagcctggccttcatccggaagagcgacgagctgctgcacaacgtgaatgctggcaagtccaccaccaacatcatgatcacaactatcatcatcgtgatcatcgtgatcctgttgagcctcatcgccgtgggcctgctgctgtattgcaaggctaggtccacccccgtgacactgtctaaggatcagctgagcggcatcaacaatatcgccttttccaactgactcgagctggtactgcatgcacgcaatgctagctgcccctttcccgtcctgggtaccccgagtctcccccacctcgggtcccaggtatgctcccacctccacctgccccactcaccacctctgctagttccagacacctcccaagcacgcagcaatgcagctcaaaacgcttagcctagccacacccccacgggaaacagcagtgattaacctttagcaataaacgaaagtttaactaagctatactaaccccagggttggtcaatttcgtgccagccacaccctggagctagcggat

SEQ ID NO: 2 - protein, 574 aa, synthetic construct
MELLILKANAITTILTAVTFCFASGQNITEEFYQSTCSAVSKGYLSALRTGWYTSVITIELSNIKENKCNGTDAKVKLIKQELDKYKNAVTELQLLMQSTPPCNNRARRELPRFMNYTLNNAKKTNVTLSKKRKRRFLGFLLGVGSACASGVAVSKVLHLEGEVNKIKSALLSTNKAVVSLSNGVSVLTIKVLDLKNYIDKQLLPIVNKQSCSISNIETVIEFQQKNNRLLEITREFSVNAGVTTPVSTYMLTNSELLSLINDMPITNDQKKLMSNNVQIVRQQSYSIMSIIKEEVLAYVVQLPLYGVIDTPCWKLHTSPLCTTNTKEGSNICLTRTDRGWYCDNAGSVSFFPQAETCKVQSNRVFCDTMNSLTLPSEINLCNVDIFNPKYDCKIMTSKTDVSSSVITSLGAIVSCYGKTKCTASNKNRGIIKTFSNGCDYVSNKGMDTVSVGNTLYYVNKQEGKSLYVKGEPIINFYDPLVFPSSEFDASISQVNEKINQSLAFIRKSDELLHNVNAGKSTTNIMITTIIIVIIVILLSLIAVGLLLYCKARSTPVTLSKDQLSGINNIAFSN